European Patent Application EP 4 230 722 A1, published August 23, 2023. Title: Bacillota strains with improved outgrowth. Applicant: Evonik Operations GmbH. The sequence listing filed with the application follows.

SEQUENCE LISTING (5 sequences)

SEQ ID NO: 1 - DNA, 1227 bp, Bacillus velezensis
  CDS (1)..(1227)
atgaaaagacgtaaatggatgcttatcctttgtacgatggtttcccttatgtttgtatccggatgctgggataaaagggagctgaccgatctagcggtgatctccgccatcggtattgaccgaaccgaaacgggaaaatacgtccttcacttgcaaattatcaatccgggaaacgtggccggcggtctgcagggcggcggagcgggagaccggcctccggtttccgtctattcggtgtccggagacaatatgacggaagctttgagaaaaggctcgatgaaagtgtccagaaggctctattttgcgcatacgaatctcgtggtgttcagtgaaaaactggcgaaagaggaagggctcagttttattctggacaatcttgaccgcgacaccgaattcaggacgaccgcaaccgttgtgatcgcgcataattgcaaggctgaagacattattaaagtgctgacgccgattgataaaatcccttccaataaagtgaacaagacgctcagcttcacgcaggaacaatacggcagagtcattaaaaccaaccttcaggacgttctgattgatctcgcttctccgaccgggtcgccgtttattccgggttatgaaatgcacggagacgataaagccggtcctacgatggaaaatacgcagacaactgaaccgaaagcagtgctgtcagcggacggactggcggtgttcaaaaaggatgggaggctggattactggattgaggatgacgacagtgtaggggctgtatggctgctcaataggatcaagcatacgttcatcaatgcggattggaagaacgtgaagcatgcaatcagtctgcaggtcacccgccagaatacaaaggtgacggccacttttccgaacggaaaaccgcatattcacgtgcatgctcaggtcgaggggctggtggacgctgtcagataccctttccatctgtctgatccgcaagtgctgatgacgatgcaaaaggcgctcagtgtgcagcttgagaaagatatcaccaaatcgattgaagatataaaagcccataagaatgacttcgtcggcttcggagacctgatctatcggaagcatccggacaaatggaaaaagttcaaagggaagtgggatgaagaatatttccccaatctccccgtagatgtcaaaacagaagtcattatcagaagaacgggcttgcggaataatcctctctcagacaagcttgagcatgattga

SEQ ID NO: 2 - protein, 408 aa, Bacillus velezensis
MKRRKWMLILCTMVSLMFVSGCWDKRELTDLAVISAIGIDRTETGKYVLHLQIINPGNVAGGLQGGGAGDRPPVSVYSVSGDNMTEALRKGSMKVSRRLYFAHTNLVVFSEKLAKEEGLSFILDNLDRDTEFRTTATVVIAHNCKAEDIIKVLTPIDKIPSNKVNKTLSFTQEQYGRVIKTNLQDVLIDLASPTGSPFIPGYEMHGDDKAGPTMENTQTTEPKAVLSADGLAVFKKDGRLDYWIEDDDSVGAVWLLNRIKHTFINADWKNVKHAISLQVTRQNTKVTATFPNGKPHIHVHAQVEGLVDAVRYPFHLSDPQVLMTMQKALSVQLEKDITKSIEDIKAHKNDFVGFGDLIYRKHPDKWKKFKGKWDEEYFPNLPVDVKTEVIIRRTGLRNNPLSDKLEHD

SEQ ID NO: 3 - DNA, 1227 bp, Bacillus velezensis
  CDS (1)..(1227)
atgaaaagacgtaaatggatgcttatccttggtacgatggtttcccttatgtttgtatccggatgctgggataaaagggagctgaccgatctagcggtgatctccgccatcggtattgaccgaaccgaaacgggaaaatacgtccttcacttgcaaattatcaatccgggaaacgtggccggcggtctgcagggcggcggagcgggagaccggtctccggtttccgtctattcggtgtccggagacaatatgacggaagctttgagaaaaggctcgatgaaagtgtccagaaggctctattttgcgcatacgaatctcgtggtgttcagtgaaaaactggcgaaagaggaagggctcagttttattctggacaatcttgaccgcgacaccgaattcaggacgaccgcaaccgttgtgatcgcgcataattgcaaggctgaagacattattaaagtgctgacgccgattgataaaatcccttccaataaagtgaacaagacgctcagcttcacgcaggaacaatacggcagagtcattaaaaccaaccttcaggacgttctgattgatctcgcttctccgaccgggtcgccgtttattccgggttatgaaatgcacggagacgataaagccggtcctacgatggaaaatacgcagacaactgaaccgaaagcagtgctgtcagcggacggactggcggtgttcaaaaaggatgggaggctggattactggattgaggatgacgacagtgtaggggctgtatggctgctcaataggatcaagcatacgttcatcaatgcggattggaagaacgtgaagcatgcaatcagtctgcaggtcacccgccagaatacaaaggtgacggccacttttccgaacggaaaaccgcatattcacgtgcatgctcaggtcgaggggctggtggacgctgtcagataccctttccatctgtctgatccgcaagtgctgatgacgatgcaaaaggcgctcagtgtgcagcttgagaaagatatcaccaaatcgattgaagatataaaagcccataagaatgacttcgtcggcttcggagacctgatctatcggaagcatccggacaaatggaaaaagttcaaagggaagtgggatgaagaatatttccccaatctccccgtagatgtcaaaacagaagtcattatcagaagaacgggcttgcggaataatcctctctcagacaagcttgagcatgattga

SEQ ID NO: 4 - protein, 408 aa, Bacillus velezensis
MKRRKWMLILGTMVSLMFVSGCWDKRELTDLAVISAIGIDRTETGKYVLHLQIINPGNVAGGLQGGGAGDRSPVSVYSVSGDNMTEALRKGSMKVSRRLYFAHTNLVVFSEKLAKEEGLSFILDNLDRDTEFRTTATVVIAHNCKAEDIIKVLTPIDKIPSNKVNKTLSFTQEQYGRVIKTNLQDVLIDLASPTGSPFIPGYEMHGDDKAGPTMENTQTTEPKAVLSADGLAVFKKDGRLDYWIEDDDSVGAVWLLNRIKHTFINADWKNVKHAISLQVTRQNTKVTATFPNGKPHIHVHAQVEGLVDAVRYPFHLSDPQVLMTMQKALSVQLEKDITKSIEDIKAHKNDFVGFGDLIYRKHPDKWKKFKGKWDEEYFPNLPVDVKTEVIIRRTGLRNNPLSDKLEHD

SEQ ID NO: 5 - DNA, 1227 bp, Bacillus velezensis
  misc_feature (6)..(6): n is a, c, g, or t
  misc_feature (21)..(21): n is a, c, g, or t
  misc_feature (24)..(25): n is a, c, g, or t
  misc_feature (46)..(46): n is a, c, g, or t
  misc_feature (48)..(49): n is a, c, g, or t
  misc_feature (58)..(58): n is a, c, g, or t
  misc_feature (63)..(63): n is a, c, g, or t
  misc_feature (66)..(66): n is a, c, g, or t
  misc_feature (78)..(78): n is a, c, g, or t
  misc_feature (84)..(84): n is a, c, g, or t
  misc_feature (87)..(87): n is a, c, g, or t
  misc_feature (91)..(91): n is a, c, g, or t
  misc_feature (93)..(93): n is a, c, g, or t
  misc_feature (96)..(96): n is a, c, g, or t
  misc_feature (102)..(102): n is a, c, g, or t
  misc_feature (108)..(108): n is a, c, g, or t
  misc_feature (123)..(123): n is a, c, g, or t
  misc_feature (126)..(126): n is a, c, g, or t
  misc_feature (130)..(130): n is a, c, g, or t
  misc_feature (138)..(138): n is a, c, g, or t
  misc_feature (141)..(141): n is a, c, g, or t
  misc_feature (144)..(145): n is a, c, g, or t
  misc_feature (150)..(150): n is a, c, g, or t
  misc_feature (153)..(153): n is a, c, g, or t
  misc_feature (165)..(165): n is a, c, g, or t
  misc_feature (168)..(168): n is a, c, g, or t
  misc_feature (174)..(174): n is a, c, g, or t
  misc_feature (183)..(183): n is a, c, g, or t
  misc_feature (189)..(189): n is a, c, g, or t
  misc_feature (214)..(214): n is a, c, g, or t
  misc_feature (216)..(216): n is a, c, g, or t
  misc_feature (234)..(234): n is a, c, g, or t
  misc_feature (237)..(237): n is a, c, g, or t
  misc_feature (250)..(250): n is a, c, g, or t
  misc_feature (273)..(275): n is a, c, g, or t
  misc_feature (282)..(282): n is a, c, g, or t
  misc_feature (291)..(291): n is a, c, g, or t
  misc_feature (300)..(300): n is a, c, g, or t
  misc_feature (306)..(306): n is a, c, g, or t
  misc_feature (312)..(312): n is a, c, g, or t
  misc_feature (318)..(318): n is a, c, g, or t
  misc_feature (336)..(336): n is a, c, g, or t
  misc_feature (358)..(359): n is a, c, g, or t
  misc_feature (366)..(367): n is a, c, g, or t
  misc_feature (384)..(384): n is a, c, g, or t
  misc_feature (390)..(390): n is a, c, g, or t
  misc_feature (405)..(405): n is a, c, g, or t
  misc_feature (411)..(411): n is a, c, g, or t
  misc_feature (413)..(414): n is a, c, g, or t
  misc_feature (417)..(417): n is a, c, g, or t
  misc_feature (420)..(420): n is a, c, g, or t
  misc_feature (423)..(423): n is a, c, g, or t
  misc_feature (431)..(431): n is a, c, g, or t
  misc_feature (438)..(438): n is a, c, g, or t
  misc_feature (450)..(450): n is a, c, g, or t
  misc_feature (462)..(462): n is a, c, g, or t
  misc_feature (504)..(504): n is a, c, g, or t
  misc_feature (510)..(510): n is a, c, g, or t
  misc_feature (531)..(531): n is a, c, g, or t
  misc_feature (543)..(543): n is a, c, g, or t
  misc_feature (545)..(546): n is a, c, g, or t
  misc_feature (573)..(573): n is a, c, g, or t
  misc_feature (580)..(581): n is a, c, g, or t
  misc_feature (588)..(588): n is a, c, g, or t
  misc_feature (597)..(597): n is a, c, g, or t
  misc_feature (600)..(600): n is a, c, g, or t
  misc_feature (607)..(607): n is a, c, g, or t
  misc_feature (621)..(622): n is a, c, g, or t
  misc_feature (624)..(624): n is a, c, g, or t
  misc_feature (629)..(629): n is a, c, g, or t
  misc_feature (633)..(633): n is a, c, g, or t
  misc_feature (639)..(639): n is a, c, g, or t
  misc_feature (657)..(657): n is a, c, g, or t
  misc_feature (667)..(667): n is a, c, g, or t
  misc_feature (672)..(673): n is a, c, g, or t
  misc_feature (675)..(675): n is a, c, g, or t
  misc_feature (684)..(684): n is a, c, g, or t
  misc_feature (691)..(691): n is a, c, g, or t
  misc_feature (696)..(696): n is a, c, g, or t
  misc_feature (699)..(699): n is a, c, g, or t
  misc_feature (711)..(711): n is a, c, g, or t
  misc_feature (714)..(714): n is a, c, g, or t
  misc_feature (717)..(717): n is a, c, g, or t
  misc_feature (720)..(720): n is a, c, g, or t
  misc_feature (732)..(733): n is a, c, g, or t
  misc_feature (739)..(739): n is a, c, g, or t
  misc_feature (741)..(741): n is a, c, g, or t
  misc_feature (750)..(750): n is a, c, g, or t
  misc_feature (753)..(753): n is a, c, g, or t
  misc_feature (756)..(756): n is a, c, g, or t
  misc_feature (768)..(768): n is a, c, g, or t
  misc_feature (771)..(771): n is a, c, g, or t
  misc_feature (773)..(774): n is a, c, g, or t
  misc_feature (780)..(780): n is a, c, g, or t
  misc_feature (810)..(810): n is a, c, g, or t
  misc_feature (813)..(813): n is a, c, g, or t
  misc_feature (819)..(819): n is a, c, g, or t
  misc_feature (822)..(822): n is a, c, g, or t
  misc_feature (843)..(843): n is a, c, g, or t
  misc_feature (852)..(852): n is a, c, g, or t
  misc_feature (855)..(855): n is a, c, g, or t
  misc_feature (874)..(876): n is a, c, g, or t
  misc_feature (879)..(879): n is a, c, g, or t
  misc_feature (886)..(886): n is a, c, g, or t
  misc_feature (897)..(897): n is a, c, g, or t
  misc_feature (904)..(904): n is a, c, g, or t
  misc_feature (909)..(909): n is a, c, g, or t
  misc_feature (912)..(912): n is a, c, g, or t
  misc_feature (915)..(917): n is a, c, g, or t
  misc_feature (927)..(928): n is a, c, g, or t
  misc_feature (933)..(933): n is a, c, g, or t
  misc_feature (936)..(936): n is a, c, g, or t
  misc_feature (942)..(942): n is a, c, g, or t
  misc_feature (958)..(958): n is a, c, g, or t
  misc_feature (969)..(969): n is a, c, g, or t
  misc_feature (971)..(973): n is a, c, g, or t
  misc_feature (990)..(990): n is a, c, g, or t
  misc_feature (992)..(993): n is a, c, g, or t
  misc_feature (1002)..(1002): n is a, c, g, or t
  misc_feature (1011)..(1011): n is a, c, g, or t
  misc_feature (1020)..(1020): n is a, c, g, or t
  misc_feature (1032)..(1032): n is a, c, g, or t
  misc_feature (1035)..(1036): n is a, c, g, or t
  misc_feature (1038)..(1038): n is a, c, g, or t
  misc_feature (1040)..(1040): n is a, c, g, or t
  misc_feature (1050)..(1050): n is a, c, g, or t
  misc_feature (1054)..(1054): n is a, c, g, or t
  misc_feature (1062)..(1062): n is a, c, g, or t
  misc_feature (1065)..(1065): n is a, c, g, or t
  misc_feature (1068)..(1068): n is a, c, g, or t
  misc_feature (1074)..(1074): n is a, c, g, or t
  misc_feature (1080)..(1081): n is a, c, g, or t
  misc_feature (1086)..(1086): n is a, c, g, or t
  misc_feature (1089)..(1090): n is a, c, g, or t
  misc_feature (1092)..(1092): n is a, c, g, or t
  misc_feature (1107)..(1108): n is a, c, g, or t
  misc_feature (1111)..(1111): n is a, c, g, or t
  misc_feature (1122)..(1122): n is a, c, g, or t
  misc_feature (1129)..(1131): n is a, c, g, or t
  misc_feature (1134)..(1134): n is a, c, g, or t
  misc_feature (1137)..(1137): n is a, c, g, or t
  misc_feature (1146)..(1146): n is a, c, g, or t
  misc_feature (1149)..(1149): n is a, c, g, or t
  misc_feature (1155)..(1155): n is a, c, g, or t
  misc_feature (1159)..(1159): n is a, c, g, or t
  misc_feature (1161)..(1161): n is a, c, g, or t
  misc_feature (1167)..(1167): n is a, c, g, or t
  misc_feature (1170)..(1170): n is a, c, g, or t
  misc_feature (1187)..(1188): n is a, c, g, or t
  misc_feature (1203)..(1203): n is a, c, g, or t
  misc_feature (1210)..(1210): n is a, c, g, or t
  misc_feature (1215)..(1216): n is a, c, g, or t
atgaanagacgtaaatggatnctnntcctttgtacgatggtttccntnntgtttgtanccggntgntgggataaaagngagctnacngatntngcngtgatntccgcnatcggtattgaccgnacngaancgggaaantangtnnttcanttncaaattatcaanccnggaaangtggccggnggtctncagggcggcggagcgggagaccggncnccggtttccgtctattcngtntccggagacaatntgacggaagctttgagaaaaggnnngatgaangtgtccagnaggctctantttgcncatacnaatctngtggtgttcagtgaaaanctggcgaaagaggaagggctcnnttttatnntggacaatcttgaccgngacacngaattcaggacgacngcaacngnngtnatngcncataattncaaggcngaagacattatnaaagtgctgacnccgattgataaaatcccttccaataaagtgaacaagacgctnagcttnacgcaggaacaatacggcagngtcattaaaacnanncttcaggacgttctgattgatctcgcntctccgnncgggtcnccgtttatnccnggttatnaaatgcacggagannanaaagncggncctacnatggaaaatacgcagacnactgaaccgnaagcnntnctgtcagcngacggantggcngtnttcaaaaagganggnagnctngattactggatnnaggatnangacagtgtnggngcngtatggctgctnaanannatcaancatacgttcatcaatgcggattggaagaangtnaagcangcnatcagtctgcaggtcacccgncagaatacnaangtgacggccacttttccgnnnggnaaaccgnatattcacgtncatgctnaggtnganggnnnggtggacgcnntcagntancctttncatctgtctgatccgnaagtgctgatnannntgcaaaaggcgctcagngnncagcttganaaagatatnaccaaatcnattgaagatatnaanncncntaagaatganttcntcggcttnggnganctgatntatcgnnagcanccnnanaaatggaaaaagttnnaanggaagtgggangaagaannnttnccnaatctcccngtngatgtnaaancngaagtnatnatcagaagaacgggctnncggaataatcctctntcagacnagctnnagcatgattga